European Patent Specification EP 3 512 869 B1, published February 28, 2024. Title: Magnetic particle-binding peptides. Applicant: Technische Universität München Karlsruher Institut für Technologie. The sequence listing filed with the application follows.

SEQUENCE LISTING (19 sequences)

SEQ ID NO: 1 - protein, 6 aa, Artificial Sequence
  iron oxide-binding peptide
EEEEEE

SEQ ID NO: 2 - protein, 6 aa, Artificial Sequence
  iron oxide-binding peptide
DDDDDD

SEQ ID NO: 3 - protein, 12 aa, Artificial Sequence
  iron oxide-binding peptide
DDDDEDDEDDDD

SEQ ID NO: 4 - protein, 12 aa, Artificial Sequence
  iron oxide-binding peptide
DDDEDDEDDEDD

SEQ ID NO: 5 - protein, 10 aa, Artificial Sequence
  iron oxide-binding peptide
DDDDDDDDDD

SEQ ID NO: 6 - protein, 12 aa, Artificial Sequence
  iron oxide-binding peptide
DDDDDEDDDDDD

SEQ ID NO: 7 - protein, 10 aa, Artificial Sequence
  iron oxide-binding peptide
DDDEDDEDDD

SEQ ID NO: 8 - protein, 12 aa, Artificial Sequence
  iron oxide-binding peptide
DDDDDDDDDDDD

SEQ ID NO: 9 - protein, 10 aa, Artificial Sequence
  iron oxide-binding peptide
DDEDDEDDED

SEQ ID NO: 10 - protein, 10 aa, Artificial Sequence
  iron oxide-binding peptide
DDDDEDDDDD

SEQ ID NO: 11 - protein, 12 aa, Artificial Sequence
  iron oxide-binding peptide
DDDDDGGDDDDD

SEQ ID NO: 12 - protein, 8 aa, Artificial Sequence
  iron oxide-binding peptide
DDDDDDDD

SEQ ID NO: 13 - protein, 10 aa, Artificial Sequence
  iron oxide-binding peptide
DDDDGGDDDD

SEQ ID NO: 14 - protein, 12 aa, Artificial Sequence
  iron oxide-binding peptide
DDDDGGGGDDDD

SEQ ID NO: 15 - protein, 10 aa, Artificial Sequence
  iron oxide-binding peptide
DDDGGGGDDD

SEQ ID NO: 16 - protein, 8 aa, Artificial Sequence
  iron oxide-binding peptide
DDDGGDDD

SEQ ID NO: 17 - protein, 12 aa, Artificial Sequence
  iron oxide-binding peptide
DDDGGGGGGDDD

SEQ ID NO: 18 - protein, 11 aa, Artificial Sequence
  iron oxide-binding peptide
DDDDDDDDDDD

SEQ ID NO: 19 - protein, 12 aa, Artificial Sequence
  iron oxide-binding peptide
EEEEGGGGEEEE